European Patent Application EP 4 234 714 A1, published August 30, 2023. Title: MULTIPLEXED SYSTEM FOR THE DETECTION OF DISEASE-RELATED microRNAS IN BIOLOGICAL SAMPLES. Applicant: Fundación IMDEA Nanociencia. The sequence listing filed with the application follows.

SEQUENCE LISTING (24 sequences)

SEQ ID NO: 1 - DNA, 22 bp, Artificial Sequence
  Probe specific for miRNA-146a
aacccatggaattcagttctca

SEQ ID NO: 2 - DNA, 23 bp, Artificial Sequence
  Probe specific for miRNA-155
acccctatcacgattagcattaa

SEQ ID NO: 3 - DNA, 21 bp, Artificial Sequence
  Probe specific for miRNA-191
agctgcttttgggattccgtt

SEQ ID NO: 4 - RNA, 22 nt, Homo sapiens
ugagaacugaauuccauggguu

SEQ ID NO: 5 - RNA, 23 nt, Homo sapiens
uuaaugcuaaucgugauaggggu

SEQ ID NO: 6 - RNA, 23 nt, Homo sapiens
caacggaaucccaaaagcagcug

SEQ ID NO: 7 - DNA, 21 bp, Artificial Sequence
  RNA Scramble Sequence R-1
uguagagaugcgguggucctt

SEQ ID NO: 8 - DNA, 21 bp, Artificial Sequence
  RNA Scramble Sequence R-2
acaucucuacgccaccaggtt

SEQ ID NO: 9 - DNA, 21 bp, Artificial Sequence
  RNA Scramble Sequence R-3
gucuccgaacgugucacgutt

SEQ ID NO: 10 - DNA, 21 bp, Artificial Sequence
  RNA Scramble Sequence R-4
cuacgccaucagcuccaactt

SEQ ID NO: 11 - RNA, 21 nt, Artificial Sequence
  RNA Scramble Sequence R-5
aagacgggagaagagaaggga

SEQ ID NO: 12 - RNA, 23 nt, Artificial Sequence
  RNA Scramble Sequence R-6
uuauugcuuaagaauacgcguag

SEQ ID NO: 13 - DNA, 22 bp, Artificial Sequence
  DNA Target Sequence T-146a
tgagaactgaattccatgggtt

SEQ ID NO: 14 - DNA, 23 bp, Artificial Sequence
  DNA Target Sequence T-155
ttaatgctaatcgtgataggggt

SEQ ID NO: 15 - DNA, 23 bp, Artificial Sequence
  DNA Target Sequence T-191
caacggaatcccaaaagcagctg

SEQ ID NO: 16 - DNA, 24 bp, Artificial Sequence
  DNA Scramble Sequence D-1
catcttcggcaaccagatcatccc

SEQ ID NO: 17 - DNA, 22 bp, Artificial Sequence
  DNA Scramble Sequence D-2
tctctgaccttaggccccctac

SEQ ID NO: 18 - DNA, 27 bp, Artificial Sequence
  DNA Scramble Sequence D-3
gaggttaacagagtgacagatggtgca

SEQ ID NO: 19 - DNA, 22 bp, Artificial Sequence
  DNA Scramble Sequence D-4
tggaatgtaaagaagtatgtat

SEQ ID NO: 20 - DNA, 21 bp, Artificial Sequence
  DNA Scramble Sequence D-5
aagacgggagaagagaaggga

SEQ ID NO: 21 - DNA, 27 bp, Artificial Sequence
  DNA Scramble Sequence D-6
acgatacagagaagattagcatggccc

SEQ ID NO: 22 - DNA, 37 bp, Artificial Sequence
  Hairpin Oligonucleotide Probe MB-146a
tttttcggccaacccatggaattcagttctcaggccg

SEQ ID NO: 23 - DNA, 38 bp, Artificial Sequence
  Hairpin Oligonucleotide Probe MB-155
tttttcggccacccctatcacgattagcattaaggccg

SEQ ID NO: 24 - DNA, 36 bp, Artificial Sequence
  Hairpin Oligonucleotide Probe MB-191
tttttggcccagctgcttttgggattccgttgggcc